European Patent Application EP 4 722 251 A1, published April 8, 2026. Title: 特异性结合的抗TFPI抗体及其用途. Applicant: 安源医药科技（上海）有限公司. The sequence listing filed with the application follows.

SEQUENCE LISTING (90 sequences)

SEQ ID NO: 1 - protein, 276 aa, Homo sapiens
DSEEDEEHTIITDTELPPLKLMHSFCAFKADDGPCKAIMKRFFFNIFTRQCEEFIYGGCEGNQNRFESLEECKKMCTRDNANRIIKTTLQQEKPDFCFLEEDPGICRGYITRYFYNNQTKQCERFKYGGCLGNMNNFETLEECKNICEDGPNGFQVDNYGTQLNAVNNSLTPQSTKVPSLFEFHGPSWCLTPADRGLCRANENRFYYNSVIGKCRPFKYSGCGGNENNFTSKQECLRACKKGFIQRISKGGLIKTKRKRKKQRVKIAYEEIFVKNM

SEQ ID NO: 2 - protein, 119 aa, synthetic construct
EVQLVQSGAELKKPGASVKLSCKASGYTFTSYWMHWVRQTPGQGLEWIGEIKPDQGRINYNEKFKTRATLTADKSTSTAYMELSSLRSEDTAVYYCARSSVVDVAMDYWGQGTTVTVSS

SEQ ID NO: 3 - protein, 108 aa, synthetic construct
EIVLTQSPATLSLSPGERATLSCSASSSVSSSYLYWYQQKPGQAPRLWISGTSILASGVPARFSGSGSGTKYTLTISSLEPEDFAVYFCHQWSHYPFTFGQGTKLEIK

SEQ ID NO: 4 - protein, 119 aa, synthetic construct
EVQLVQSGAELKKPGASVKLSCKASGYTFTSYWMHWVRQAPGQGLEWIGEIKPDQGRINYNEKFKTRATLTADKSTSTAYMELSSLRSEDTAVYYCARSSHVDVAMDYWGQGTTVTVSS

SEQ ID NO: 5 - protein, 108 aa, synthetic construct; identical to SEQ ID NO: 3

SEQ ID NO: 6 - protein, 119 aa, synthetic construct
EVQLVQSGAELKKPGASVKLSCKASGYTFTSYWMHWVRQAPGQGLEWIGEIKPDQGRINYNEKFKTRATLTADKSTSTAYMELSSLRSEDTAVYYCARSSVIDVAMDYWGQGTTVTVSS

SEQ ID NO: 7 - protein, 108 aa, synthetic construct; identical to SEQ ID NO: 3

SEQ ID NO: 8 - protein, 119 aa, synthetic construct
EVQLVQSGAELKKPGASVKLSCKASGYTFTSYWMHWVRQAPGQGLEWIGEIKPDQGRIHYNEKFKTRATLTADKSTSTAYMELSSLRSEDTAVYYCARSSVVDVAMDYWGQGTTVTVSS

SEQ ID NO: 9 - protein, 108 aa, synthetic construct; identical to SEQ ID NO: 3

SEQ ID NO: 10 - protein, 119 aa, synthetic construct
EVQLVQSGAELKKPGASVKLSCKASGYTFTSYWMHWVRQAPGQGLEWIGEIKPDHGRINYNEKFKTRATLTADKSTSTAYMELSSLRSEDTAVYYCARSSVVDVAMDYWGQGTTVTVSS

SEQ ID NO: 11 - protein, 108 aa, synthetic construct; identical to SEQ ID NO: 3

SEQ ID NO: 12 - protein, 119 aa, synthetic construct
EVQLVQSGAELKKPGASVKLSCKASGYTFTSYWMHWVRQAPGQGLEWIGEIKPDKGRINYNEKFKTRATLTADKSTSTAYMELSSLRSEDTAVYYCARSSVVDVAMDYWGQGTTVTVSS

SEQ ID NO: 13 - protein, 108 aa, synthetic construct; identical to SEQ ID NO: 3

SEQ ID NO: 14 - protein, 119 aa, synthetic construct
EVQLVQSGAELKKPGASVKLSCKASGYTFTSYWMHWVRQAPGQGLEWIGEIKPDQGRIDYNEKFKTRATLTADKSTSTAYMELSSLRSEDTAVYYCARSSVVDVAMDYWGQGTTVTVSS

SEQ ID NO: 15 - protein, 108 aa, synthetic construct; identical to SEQ ID NO: 3

SEQ ID NO: 16 - protein, 119 aa, synthetic construct
EVQLVQSGAELKKPGASVKLSCKASGYTFTSYWMHWVRQAPGQGLEWIGEIKPDQGRINYNEKFKTRATLTADKSTSTAYMELSSLRSEDTAVYYCARSSVVDVAMDYWGQGTTVTVSS

SEQ ID NO: 17 - protein, 108 aa, synthetic construct
EIVLTQSPATLSLSPGERATLSCSASSSVSSSYLYWYQQKPGQAPRLWISGTSILASGVPARFSGSGSGTKYTLTISSLEPEDFAVYFCHQWSYYPFTFGQGTKLEIK

SEQ ID NO: 18 - protein, 119 aa, synthetic construct; identical to SEQ ID NO: 16

SEQ ID NO: 19 - protein, 108 aa, synthetic construct
EIVLTQSPATLSLSPGERATLSCSASSSVSSSYLYWYQQKPGQAPRLWISGTSILASGVPARFSGSGSGTKYTLTISSLEPEDFAVYFCHQWSFYPFTFGQGTKLEIK

SEQ ID NO: 20 - protein, 119 aa, synthetic construct; identical to SEQ ID NO: 16

SEQ ID NO: 21 - protein, 108 aa, synthetic construct
EIVLTQSPATLSLSPGERATLSCSASSSVSSSYLYWYQQKPGQAPRLWISGTSILASGVPARFSGSGSGTKYTLTISSLEPEDFAVYFCHQWTHYPFTFGQGTKLEIK

SEQ ID NO: 22 - protein, 119 aa, synthetic construct
EVQLVQSGAELKKPGASVKLSCKASGYTFTSYWMHWVRQAPGQGLEWIGEIKPDKGRINYNEKFKTRATLTADKSTSTAYMELSSLRSEDTAVYYCARSSVIDVAMDYWGQGTTVTVSS

SEQ ID NO: 23 - protein, 108 aa, synthetic construct; identical to SEQ ID NO: 3

SEQ ID NO: 24 - protein, 119 aa, synthetic construct
EVQLVQSGAELKKPGASVKLSCKASGYTFTSYWMHWVRQAPGQGLEWIGEIKPDQGRINYNEKFKTRATLTADKSTSTAYMELSSLRSEDTAVYYCARSSVVDDAMDYWGQGTTVTVSS

SEQ ID NO: 25 - protein, 108 aa, synthetic construct; identical to SEQ ID NO: 3

SEQ ID NO: 26 - protein, 119 aa, synthetic construct
EVQLVQSGAELKKPGASVKLSCKASGYTFTSYWMHWVRQAPGQGLEWIGEIKPDQGRINYNEKFKTRATLTADKSTSTAYMELSSLRSEDTAVYYCARSSVVDTAMDYWGQGTTVTVSS

SEQ ID NO: 27 - protein, 108 aa, synthetic construct; identical to SEQ ID NO: 3

SEQ ID NO: 28 - protein, 119 aa, synthetic construct
EVQLVQSGAELKKPGASVKLSCKASGYTFTSYWMHWVRQAPGQGLEWIGEIKPDQGRINYNEKFKTRATLTADKSTSTAYMELSSLRSEDTAVYYCARSSVVDEAMDYWGQGTTVTVSS

SEQ ID NO: 29 - protein, 108 aa, synthetic construct; identical to SEQ ID NO: 3

SEQ ID NO: 30 - protein, 119 aa, synthetic construct
EVQLVQSGAELKKPGASVKLSCKASGYTFTSYWMHWVRQAPGQGLEWIGEIKPDQGRINYNEKFKTRATLTADKSTSTAYMELSSLRSEDTAVYYCARSSVVDVALDYWGQGTTVTVSS

SEQ ID NO: 31 - protein, 108 aa, synthetic construct; identical to SEQ ID NO: 3

SEQ ID NO: 32 - protein, 119 aa, synthetic construct
EVQLVQSGAELKKPGASVKLSCKASGYTFTSYWMHWVRQAPGQGLEWIGEIKPDQGRINYNEKFKTRATLTADKSTSTAYMELSSLRSEDTAVYYCARSSVVDVAIDYWGQGTTVTVSS

SEQ ID NO: 33 - protein, 108 aa, synthetic construct; identical to SEQ ID NO: 3

SEQ ID NO: 34 - protein, 119 aa, synthetic construct
EVQLVQSGAELKKPGASVKLSCKASGYTFTSYWMHWVRQAPGQGLEWIGEIKPDQGRINYNEKFKTRATLTADKSTSTAYMELSSLRSEDTAVYYCARSSVVDVAEDYWGQGTTVTVSS

SEQ ID NO: 35 - protein, 108 aa, synthetic construct; identical to SEQ ID NO: 3

SEQ ID NO: 36 - protein, 119 aa, synthetic construct
EVQLVQSGAELKKPGASVKLSCKASGYTFTSYWMHWVRQAPGQGLEWIGEIKPDQGRINYNEKFKTRATLTADKSTSTAYMELSSLRSEDTAVYYCARSSVVDVAVDYWGQGTTVTVSS

SEQ ID NO: 37 - protein, 108 aa, synthetic construct; identical to SEQ ID NO: 3

SEQ ID NO: 38 - protein, 119 aa, synthetic construct
EVQLVQSGAELKKPGASVKLSCKASGYTFTSYWMHWVRQAPGQGLEWIGEIKPDQGRINYNEKFKTRATLTADKSTSTAYMELSSLRSEDTAVYYCARSSVVDVADDYWGQGTTVTVSS

SEQ ID NO: 39 - protein, 108 aa, synthetic construct; identical to SEQ ID NO: 3

SEQ ID NO: 40 - protein, 119 aa, synthetic construct
EVQLVQSGAELKKPGASVKLSCKASGYTFTSYWMHWVRQAPGQGLEWIGEIKPDQGRINYNEKFKTRATLTADKSTSTAYMELSSLRSEDTAVYYCARSSVFDVAMDYWGQGTTVTVSS

SEQ ID NO: 41 - protein, 108 aa, synthetic construct; identical to SEQ ID NO: 3

SEQ ID NO: 42 - protein, 119 aa, synthetic construct
EVQLVQSGAELKKPGASVKLSCKASGYTFTSYWMHWVRQAPGQGLEWIGEIKPDQGRINYNEKFKTRATLTADKSTSTAYMELSSLRSEDTAVYYCARSSVYDVAMDYWGQGTTVTVSS

SEQ ID NO: 43 - protein, 108 aa, synthetic construct; identical to SEQ ID NO: 3

SEQ ID NO: 44 - protein, 119 aa, synthetic construct
EVQLVQSGAELKKPGASVKLSCKASGYTFTSYWMHWVRQAPGQGLEWIGEIKPDQGRINYNEKFKTRATLTADKSTSTAYMELSSLRSEDTAVYYCARSSVLDVAMDYWGQGTTVTVSS

SEQ ID NO: 45 - protein, 108 aa, synthetic construct; identical to SEQ ID NO: 3

SEQ ID NO: 46 - protein, 5 aa, synthetic construct
SYWMH

SEQ ID NO: 47 - protein, 17 aa, synthetic construct
EIKPDQGRINYNEKFKT

SEQ ID NO: 48 - protein, 10 aa, synthetic construct
SSVVDVAMDY

SEQ ID NO: 49 - protein, 12 aa, synthetic construct
SASSSVSSSYLY

SEQ ID NO: 50 - protein, 7 aa, synthetic construct
GTSILAS

SEQ ID NO: 51 - protein, 9 aa, synthetic construct
HQWSHYPFT

SEQ ID NO: 52 - protein, 8 aa, synthetic construct
GYTFTSYW

SEQ ID NO: 53 - protein, 8 aa, synthetic construct
IKPDQGRI

SEQ ID NO: 54 - protein, 12 aa, synthetic construct
ARSSVVDVAMDY

SEQ ID NO: 55 - protein, 7 aa, synthetic construct
SSVSSSY

SEQ ID NO: 56 - protein, 10 aa, synthetic construct
SSHVDVAMDY

SEQ ID NO: 57 - protein, 12 aa, synthetic construct
ARSSHVDVAMDY

SEQ ID NO: 58 - protein, 10 aa, synthetic construct
SSVIDVAMDY

SEQ ID NO: 59 - protein, 12 aa, synthetic construct
ARSSVIDVAMDY

SEQ ID NO: 60 - protein, 17 aa, synthetic construct
EIKPDQGRIHYNEKFKT

SEQ ID NO: 61 - protein, 17 aa, synthetic construct
EIKPDHGRINYNEKFKT

SEQ ID NO: 62 - protein, 8 aa, synthetic construct
IKPDHGRI

SEQ ID NO: 63 - protein, 17 aa, synthetic construct
EIKPDKGRINYNEKFKT

SEQ ID NO: 64 - protein, 8 aa, synthetic construct
IKPDKGRI

SEQ ID NO: 65 - protein, 17 aa, synthetic construct
EIKPDQGRIDYNEKFKT

SEQ ID NO: 66 - protein, 9 aa, synthetic construct
HQWSYYPFT

SEQ ID NO: 67 - protein, 9 aa, synthetic construct
HQWSFYPFT

SEQ ID NO: 68 - protein, 9 aa, synthetic construct
HQWTHYPFT

SEQ ID NO: 69 - protein, 10 aa, synthetic construct
SSVVDDAMDY

SEQ ID NO: 70 - protein, 12 aa, synthetic construct
ARSSVVDDAMDY

SEQ ID NO: 71 - protein, 10 aa, synthetic construct
SSVVDTAMDY

SEQ ID NO: 72 - protein, 12 aa, synthetic construct
ARSSVVDTAMDY

SEQ ID NO: 73 - protein, 10 aa, synthetic construct
SSVVDEAMDY

SEQ ID NO: 74 - protein, 12 aa, synthetic construct
ARSSVVDEAMDY

SEQ ID NO: 75 - protein, 10 aa, synthetic construct
SSVVDVALDY

SEQ ID NO: 76 - protein, 12 aa, synthetic construct
ARSSVVDVALDY

SEQ ID NO: 77 - protein, 10 aa, synthetic construct
SSVVDVAIDY

SEQ ID NO: 78 - protein, 12 aa, synthetic construct
ARSSVVDVAIDY

SEQ ID NO: 79 - protein, 10 aa, synthetic construct
SSVVDVAEDY

SEQ ID NO: 80 - protein, 12 aa, synthetic construct
ARSSVVDVAEDY

SEQ ID NO: 81 - protein, 10 aa, synthetic construct
SSVVDVAVDY

SEQ ID NO: 82 - protein, 12 aa, synthetic construct
ARSSVVDVAVDY

SEQ ID NO: 83 - protein, 10 aa, synthetic construct
SSVVDVADDY

SEQ ID NO: 84 - protein, 12 aa, synthetic construct
ARSSVVDVADDY

SEQ ID NO: 85 - protein, 10 aa, synthetic construct
SSVFDVAMDY

SEQ ID NO: 86 - protein, 12 aa, synthetic construct
ARSSVFDVAMDY

SEQ ID NO: 87 - protein, 10 aa, synthetic construct
SSVYDVAMDY

SEQ ID NO: 88 - protein, 12 aa, synthetic construct
ARSSVYDVAMDY

SEQ ID NO: 89 - protein, 10 aa, synthetic construct
SSVLDVAMDY

SEQ ID NO: 90 - protein, 12 aa, synthetic construct
ARSSVLDVAMDY